European Patent Specification EP 4 337 780 B1, published April 1, 2026. Title: Recombinant TERT-encoding viral genomes and vectors. Applicant: Fundación del Sector Público Estatal Centro Nacional de Investigaciones Oncológicas Carlos III (F.S.P. CNIO) Universitat Autònoma de Barcelona. The sequence listing filed with the application follows.

SEQUENCE LISTING (46 sequences)

SEQ ID NO: 1 - DNA, 3786 bp, Mus musculus
  mTERT CDS + native 3' UTR
atgacccgcgctcctcgttgccccgcggtgcgctctctgctgcgcagccgataccgggaggtgtggccgctggcaacctttgtgcggcgcctggggcccgagggcaggcggcttgtgcaacccggggacccgaagatctaccgcactttggttgcccaatgcctagtgtgcatgcactggggctcacagcctccacctgccgacctttccttccaccaggtgtcatccctgaaagagctggtggccagggttgtgcagagactctgcgagcgcaacgagagaaacgtgctggcttttggctttgagctgcttaacgaggccagaggcgggcctcccatggccttcactagtagcgtgcgtagctacttgcccaacactgttattgagaccctgcgtgtcagtggtgcatggatgctactgttgagccgagtgggcgacgacctgctggtctacctgctggcacactgtgctctttatcttctggtgccccccagctgtgcctaccaggtgtgtgggtctcccctgtaccaaatttgtgccaccacggatatctggccctctgtgtccgctagttacaggcccacccgacccgtgggcaggaatttcactaaccttaggttcttacaacagatcaagagcagtagtcgccaggaagcaccgaaacccctggccttgccatctcgaggtacaaagaggcatctgagtctcaccagtacaagtgtgccttcagctaagaaggccagatgctatcctgtcccgagagtggaggagggaccccacaggcaggtgctaccaaccccatcaggcaaatcatgggtgccaagtcctgctcggtcccccgaggtgcctactgcagagaaagatttgtcttctaaaggaaaggtgtctgacctgagtctctctgggtcggtgtgctgtaaacacaagcccagctccacatctctgctgtcaccaccccgccaaaatgcctttcagctcaggccatttattgagaccagacatttcctttactccaggggagatggccaagagcgtctaaacccctcattcctactcagcaacctccagcctaacttgactggggccaggagactggtggagatcatctttctgggctcaaggcctaggacatcaggaccactctgcaggacacaccgtctatcgcgtcgatactggcagatgcggcccctgttccaacagctgctggtgaaccatgcagagtgccaatatgtcagactcctcaggtcacattgcaggtttcgaacagcaaaccaacaggtgacagatgccttgaacaccagcccaccgcacctcatggatttgctccgcctgcacagcagtccctggcaggtatatggttttcttcgggcctgtctctgcaaggtggtgtctgctagtctctggggtaccaggcacaatgagcgccgcttctttaagaacttaaagaagttcatctcgttggggaaatacggcaagctatcactgcaggaactgatgtggaagatgaaagtagaggattgccactggctccgcagcagcccggggaaggaccgtgtccccgctgcagagcaccgtctgagggagaggatcctggctacgttcctgttctggctgatggacacatacgtggtacagctgcttaggtcattcttttacatcacagagagcacattccagaagaacaggctcttcttctaccgtaagagtgtgtggagcaagctgcagagcattggagtcaggcaacaccttgagagagtgcggctacgggagctgtcacaagaggaggtcaggcatcaccaggacacctggctagccatgcccatctgcagactgcgcttcatccccaagcccaacggcctgcggcccattgtgaacatgagttatagcatgggtaccagagctttgggcagaaggaagcaggcccagcatttcacccagcgtctcaagactctcttcagcatgctcaactatgagcggacaaaacatcctcaccttatggggtcttctgtactgggtatgaatgacatctacaggacctggcgggcctttgtgctgcgtgtgcgtgctctggaccagacacccaggatgtactttgttaaggcagatgtgaccggggcctatgatgccatcccccagggtaagctggtggaggttgttgccaatatgatcaggcactcggagagcacgtactgtatccgccagtatgcagtggtccggagagatagccaaggccaagtccacaagtcctttaggagacaggtcaccaccctctctgacctccagccatacatgggccagttccttaagcatctgcaggattcagatgccagtgcactgaggaactccgttgtcatcgagcagagcatctctatgaatgagagcagcagcagcctgtttgacttcttcctgcacttcctgcgtcacagtgtcgtaaagattggtgacaggtgctatacgcagtgccagggcatcccccagggctccagcctatccaccctgctctgcagtctgtgtttcggagacatggagaacaagctgtttgctgaggtgcagcgggatgggttgcttttacgttttgttgatgactttctgttggtgacgcctcacttggaccaagcaaaaaccttcctcagcaccctggtccatggcgttcctgagtatgggtgcatgataaacttgcagaagacagtggtgaacttccctgtggagcctggtaccctgggtggtgcagctccataccagctgcctgctcactgcctgtttccctggtgtggcttgctgctggacactcagactttggaggtgttctgtgactactcaggttatgcccagacctcaattaagacgagcctcaccttccagagtgtcttcaaagctgggaagaccatgcggaacaagctcctgtcggtcttgcggttgaagtgtcacggtctatttctagacttgcaggtgaacagcctccagacagtctgcatcaatatatacaagatcttcctgcttcaggcctacaggttccatgcatgtgtgattcagcttccctttgaccagcgtgttaggaagaacctcacattctttctgggcatcatctccagccaagcatcctgctgctatgctatcctgaaggtcaagaatccaggaatgacactaaaggcctctggctcctttcctcctgaagccgcacattggctctgctaccaggccttcctgctcaagctggctgctcattctgtcatctacaaatgtctcctgggacctctgaggacagcccaaaaactgctgtgccggaagctcccagaggcgacaatgaccatccttaaagctgcagctgacccagccctaagcacagactttcagaccattttggactaaccctgtctccttccgctagatgaacatgggcattgtagcctcagcactcctggatccacgtcacaagagggactggtcagttgtgaggctaggtcatcctccaaacctctgtgtcatgggtggtatgggagattgtcccagtgccttgtttcctgtaacaggcttgatttctttcctgatgccctcagggaggcagatcctatcccttttagtggcagggatccactagcaccagcacatgaggagtgcacccagtgcacatgggcactgggacagtggacaggtgtgagattcctgggccctggagtcttttcacacctaaccatggagcctgtcccagtacatcagagtgcctcggagatgaaaaaggacatcgagccagtgacctaaattacagcctgaatatactctgaattc

SEQ ID NO: 2 - DNA, 3369 bp, Artificial sequence
  mTERT CDS
atgacccgcgctcctcgttgccccgcggtgcgctctctgctgcgcagccgataccgggaggtgtggccgctggcaacctttgtgcggcgcctggggcccgagggcaggcggcttgtgcaacccggggacccgaagatctaccgcactttggttgcccaatgcctagtgtgcatgcactggggctcacagcctccacctgccgacctttccttccaccaggtgtcatccctgaaagagctggtggccagggttgtgcagagactctgcgagcgcaacgagagaaacgtgctggcttttggctttgagctgcttaacgaggccagaggcgggcctcccatggccttcactagtagcgtgcgtagctacttgcccaacactgttattgagaccctgcgtgtcagtggtgcatggatgctactgttgagccgagtgggcgacgacctgctggtctacctgctggcacactgtgctctttatcttctggtgccccccagctgtgcctaccaggtgtgtgggtctcccctgtaccaaatttgtgccaccacggatatctggccctctgtgtccgctagttacaggcccacccgacccgtgggcaggaatttcactaaccttaggttcttacaacagatcaagagcagtagtcgccaggaagcaccgaaacccctggccttgccatctcgaggtacaaagaggcatctgagtctcaccagtacaagtgtgccttcagctaagaaggccagatgctatcctgtcccgagagtggaggagggaccccacaggcaggtgctaccaaccccatcaggcaaatcatgggtgccaagtcctgctcggtcccccgaggtgcctactgcagagaaagatttgtcttctaaaggaaaggtgtctgacctgagtctctctgggtcggtgtgctgtaaacacaagcccagctccacatctctgctgtcaccaccccgccaaaatgcctttcagctcaggccatttattgagaccagacatttcctttactccaggggagatggccaagagcgtctaaacccctcattcctactcagcaacctccagcctaacttgactggggccaggagactggtggagatcatctttctgggctcaaggcctaggacatcaggaccactctgcaggacacaccgtctatcgcgtcgatactggcagatgcggcccctgttccaacagctgctggtgaaccatgcagagtgccaatatgtcagactcctcaggtcacattgcaggtttcgaacagcaaaccaacaggtgacagatgccttgaacaccagcccaccgcacctcatggatttgctccgcctgcacagcagtccctggcaggtatatggttttcttcgggcctgtctctgcaaggtggtgtctgctagtctctggggtaccaggcacaatgagcgccgcttctttaagaacttaaagaagttcatctcgttggggaaatacggcaagctatcactgcaggaactgatgtggaagatgaaagtagaggattgccactggctccgcagcagcccggggaaggaccgtgtccccgctgcagagcaccgtctgagggagaggatcctggctacgttcctgttctggctgatggacacatacgtggtacagctgcttaggtcattcttttacatcacagagagcacattccagaagaacaggctcttcttctaccgtaagagtgtgtggagcaagctgcagagcattggagtcaggcaacaccttgagagagtgcggctacgggagctgtcacaagaggaggtcaggcatcaccaggacacctggctagccatgcccatctgcagactgcgcttcatccccaagcccaacggcctgcggcccattgtgaacatgagttatagcatgggtaccagagctttgggcagaaggaagcaggcccagcatttcacccagcgtctcaagactctcttcagcatgctcaactatgagcggacaaaacatcctcaccttatggggtcttctgtactgggtatgaatgacatctacaggacctggcgggcctttgtgctgcgtgtgcgtgctctggaccagacacccaggatgtactttgttaaggcagatgtgaccggggcctatgatgccatcccccagggtaagctggtggaggttgttgccaatatgatcaggcactcggagagcacgtactgtatccgccagtatgcagtggtccggagagatagccaaggccaagtccacaagtcctttaggagacaggtcaccaccctctctgacctccagccatacatgggccagttccttaagcatctgcaggattcagatgccagtgcactgaggaactccgttgtcatcgagcagagcatctctatgaatgagagcagcagcagcctgtttgacttcttcctgcacttcctgcgtcacagtgtcgtaaagattggtgacaggtgctatacgcagtgccagggcatcccccagggctccagcctatccaccctgctctgcagtctgtgtttcggagacatggagaacaagctgtttgctgaggtgcagcgggatgggttgcttttacgttttgttgatgactttctgttggtgacgcctcacttggaccaagcaaaaaccttcctcagcaccctggtccatggcgttcctgagtatgggtgcatgataaacttgcagaagacagtggtgaacttccctgtggagcctggtaccctgggtggtgcagctccataccagctgcctgctcactgcctgtttccctggtgtggcttgctgctggacactcagactttggaggtgttctgtgactactcaggttatgcccagacctcaattaagacgagcctcaccttccagagtgtcttcaaagctgggaagaccatgcggaacaagctcctgtcggtcttgcggttgaagtgtcacggtctatttctagacttgcaggtgaacagcctccagacagtctgcatcaatatatacaagatcttcctgcttcaggcctacaggttccatgcatgtgtgattcagcttccctttgaccagcgtgttaggaagaacctcacattctttctgggcatcatctccagccaagcatcctgctgctatgctatcctgaaggtcaagaatccaggaatgacactaaaggcctctggctcctttcctcctgaagccgcacattggctctgctaccaggccttcctgctcaagctggctgctcattctgtcatctacaaatgtctcctgggacctctgaggacagcccaaaaactgctgtgccggaagctcccagaggcgacaatgaccatccttaaagctgcagctgacccagccctaagcacagactttcagaccattttggactaa

SEQ ID NO: 3 - DNA, 3369 bp, Artificial sequence
  moTERT
atgacaagagcccctagatgtcctgccgtcagaagcctgctgagaagcagatacagagaagtgtggcccctggccaccttcgtcagaaggcttggacctgaaggcagacggctggttcaacctggcgaccccaagatctacagaaccctggtggctcagtgcctcgtgtgtatgcactggggatctcagccacctcctgccgatctgagctttcaccaggtgtccagcctgaaagaactggtggccagagtggtgcagagactgtgcgagagaaacgagaggaacgtgctggccttcggcttcgagctgctgaatgaagctagaggcggccctcctatggccttcacatctagcgtgcggagctacctgcctaacaccgtgatcgagacactgagagtgtccggcgcttggatgctgctgctgagcagagtgggagatgacctgctggtgtacctgctggctcactgtgccctctatctgctggtgcctcctagctgcgcttaccaagtgtgcggaagccctctgtaccagatctgtgccaccaccgacatctggcctagcgtgtccgcttcctacagacccacaagacccgtgggcagaaactttaccaacctgagattcctgcagcagatcaagagcagctccaggcaagaggcccctaagcctcttgctctgcctagcagaggcaccaagagacacctgagcctgaccagcacaagcgtgccctctgccaagaaagccagatgctaccccgtgcctagagtggaagagggcccacatagacaggtgctgcctacacctagcggcaagagctgggttccatctcctgctagaagccctgaggtgccaacagccgagaaggacctgagcagcaagggcaaagtgtccgacctgtctctgagcggcagcgtgtgttgcaagcacaagcctagcagcaccagcctgctgtccccacctagacagaacgctttccagctgaggccctttatcgagacaagacacttcctgtacagcagaggcgacggccaagagagactgaaccctagcttcctgctgtctaacctgcagcctaacctgaccggcgctagaaggctggtggaaatcatcttcctgggcagcagacccagaaccagcggacctctgtgtagaacccacagactgagcagacggtactggcagatgaggcccctgttccagcagctcctggtcaaccatgccgagtgtcagtatgtgcggctgctgaggtcccactgcagattcagaaccgccaaccagcaagtgacagacgccctgaacacaagccctccacacctgatggatctgctgagactgcacagcagcccctggcaggtctacggctttctgagagcctgtctgtgcaaggtggtgtccgcatctctgtggggcaccagacacaacgagagaagattcttcaagaacctgaagaagttcatcagcctggggaagtacggcaagctgtccctgcaagaactgatgtggaagatgaaggtcgaggactgccactggctgaggtctagccctggcaaggatagagtgcctgccgctgagcacaggctgagagagagaatcctggccacattcctgttctggctgatggacacctacgtggtgcagctgctgcggagcttcttctacatcaccgagagcaccttccagaagaaccggctgttcttctaccgcaagagcgtgtggtccaagctgcagagcatcggcgtcagacagcacctggaaagagtgcgcctgagagagctgagccaagaggaagtgcggcaccaccaggatacctggctggccatgcctatctgcagactgagattcatccccaagcctaacggcctgaggcctatcgtgaacatgagctacagcatgggcactagagccctgggcagaagaaagcaggcccagcacttcacccagaggctgaaaaccctgttctccatgctgaactacgagcggacaaagcaccctcatctgatgggctcctctgtgctgggcatgaacgacatctacaggacctggcgggccttcgtgctgagagtcagagcactggaccagacacctagaatgtacttcgtgaaggccgacgtgacaggcgcctacgatgctatccctcagggcaaactggtggaagtggtggccaacatgatcaggcacagcgagtccacctactgcatcagacagtacgccgtcgtgcggagagactctcagggacaagtgcacaagagcttccgcagacaagtgaccacactgagcgatctgcagccctacatgggccagtttctgaagcacctccaggacagcgacgccagcgctctgagaaactctgtggtcatcgagcagtccatctccatgaacgagtccagctccagcctgttcgacttcttcctgcacttcctgcggcacagcgtggtcaagatcggcgacagatgttacacccagtgccagggcatcccacagggaagcagtctgagcacactgctgtgctccctgtgtttcggcgacatggaaaacaagctgttcgccgaagtgcagcgcgacggactgctcctgagatttgtggacgacttcctgctcgtgacccctcacctggatcaggctaagaccttcctgagcaccctggtgcatggcgtgccagagtacggctgcatgatcaacctgcagaaaaccgtggtcaacttccccgtggaacctggcactcttggaggcgctgctccttatcagctgcccgctcattgtctgttcccttggtgcggactgctgctggacacacagaccctggaagtgttctgcgactacagcggctacgcccagaccagcatcaagaccagcctgaccttccagtccgtgttcaaggccggcaagaccatgaggaacaagctgctgagtgtgctgaggctgaagtgccacggcctgtttctggacctgcaagtgaacagcctgcagaccgtgtgcatcaatatctacaagatctttctgctgcaagcctaccggttccacgcctgtgtgattcagctgcctttcgaccagagagtgcggaagaatctgacattctttctgggcatcatcagcagccaggccagctgctgttacgccatcctgaaagtgaagaaccccggcatgaccctgaaggcctctggcagctttccacctgaagctgcccattggctgtgctaccaggctttcctgctgaaactggctgcccacagcgtgatctacaagtgcctgctgggcccactgagaacagcccagaaactgctgtgtcggaagctgcctgaagccacaatgacaatcctgaaggctgccgccgatccagctctgagcaccgacttccagaccatcctggactga

SEQ ID NO: 4 - protein, 1122 aa, Mus musculus
  mTERT protein
MTRAPRCPAVRSLLRSRYREVWPLATFVRRLGPEGRRLVQPGDPKIYRTLVAQCLVCMHWGSQPPPADLSFHQVSSLKELVARVVQRLCERNERNVLAFGFELLNEARGGPPMAFTSSVRSYLPNTVIETLRVSGAWMLLLSRVGDDLLVYLLAHCALYLLVPPSCAYQVCGSPLYQICATTDIWPSVSASYRPTRPVGRNFTNLRFLQQIKSSSRQEAPKPLALPSRGTKRHLSLTSTSVPSAKKARCYPVPRVEEGPHRQVLPTPSGKSWVPSPARSPEVPTAEKDLSSKGKVSDLSLSGSVCCKHKPSSTSLLSPPRQNAFQLRPFIETRHFLYSRGDGQERLNPSFLLSNLQPNLTGARRLVEIIFLGSRPRTSGPLCRTHRLSRRYWQMRPLFQQLLVNHAECQYVRLLRSHCRFRTANQQVTDALNTSPPHLMDLLRLHSSPWQVYGFLRACLCKVVSASLWGTRHNERRFFKNLKKFISLGKYGKLSLQELMWKMKVEDCHWLRSSPGKDRVPAAEHRLRERILATFLFWLMDTYVVQLLRSFFYITESTFQKNRLFFYRKSVWSKLQSIGVRQHLERVRLRELSQEEVRHHQDTWLAMPICRLRFIPKPNGLRPIVNMSYSMGTRALGRRKQAQHFTQRLKTLFSMLNYERTKHPHLMGSSVLGMNDIYRTWRAFVLRVRALDQTPRMYFVKADVTGAYDAIPQGKLVEVVANMIRHSESTYCIRQYAVVRRDSQGQVHKSFRRQVTTLSDLQPYMGQFLKHLQDSDASALRNSVVIEQSISMNESSSSLFDFFLHFLRHSVVKIGDRCYTQCQGIPQGSSLSTLLCSLCFGDMENKLFAEVQRDGLLLRFVDDFLLVTPHLDQAKTFLSTLVHGVPEYGCMINLQKTVVNFPVEPGTLGGAAPYQLPAHCLFPWCGLLLDTQTLEVFCDYSGYAQTSIKTSLTFQSVFKAGKTMRNKLLSVLRLKCHGLFLDLQVNSLQTVCINIYKIFLLQAYRFHACVIQLPFDQRVRKNLTFFLGIISSQASCCYAILKVKNPGMTLKASGSFPPEAAHWLCYQAFLLKLAAHSVIYKCLLGPLRTAQKLLCRKLPEATMTILKAAADPALSTDFQTILD

SEQ ID NO: 5 - DNA, 3399 bp, Homo sapiens
  hTERT long isoform
atgccgcgcgctccccgctgccgagccgtgcgctccctgctgcgcagccactaccgcgaggtgctgccgctggccacgttcgtgcggcgcctggggccccagggctggcggctggtgcagcgcggggacccggcggctttccgcgcgctggtggcccagtgcctggtgtgcgtgccctgggacgcacggccgccccccgccgccccctccttccgccaggtgtcctgcctgaaggagctggtggcccgagtgctgcagaggctgtgcgagcgcggcgcgaagaacgtgctggccttcggcttcgcgctgctggacggggcccgcgggggcccccccgaggccttcaccaccagcgtgcgcagctacctgcccaacacggtgaccgacgcactgcgggggagcggggcgtgggggctgctgctgcgccgcgtgggcgacgacgtgctggttcacctgctggcacgctgcgcgctctttgtgctggtggctcccagctgcgcctaccaggtgtgcgggccgccgctgtaccagctcggcgctgccactcaggcccggcccccgccacacgctagtggaccccgaaggcgtctgggatgcgaacgggcctggaaccatagcgtcagggaggccggggtccccctgggcctgccagccccgggtgcgaggaggcgcgggggcagtgccagccgaagtctgccgttgcccaagaggcccaggcgtggcgctgcccctgagccggagcggacgcccgttgggcaggggtcctgggcccacccgggcaggacgcgtggaccgagtgaccgtggtttctgtgtggtgtcacctgccagacccgccgaagaagccacctctttggagggtgcgctctctggcacgcgccactcccacccatccgtgggccgccagcaccacgcgggccccccatccacatcgcggccaccacgtccctgggacacgccttgtcccccggtgtacgccgagaccaagcacttcctctactcctcaggcgacaaggagcagctgcggccctccttcctactcagctctctgaggcccagcctgactggcgctcggaggctcgtggagaccatctttctgggttccaggccctggatgccagggactccccgcaggttgccccgcctgccccagcgctactggcaaatgcggcccctgtttctggagctgcttgggaaccacgcgcagtgcccctacggggtgctcctcaagacgcactgcccgctgcgagctgcggtcaccccagcagccggtgtctgtgcccgggagaagccccagggctctgtggcggcccccgaggaggaggacacagacccccgtcgcctggtgcagctgctccgccagcacagcagcccctggcaggtgtacggcttcgtgcgggcctgcctgcgccggctggtgcccccaggcctctggggctccaggcacaacgaacgccgcttcctcaggaacaccaagaagttcatctccctggggaagcatgccaagctctcgctgcaggagctgacgtggaagatgagcgtgcgggactgcgcttggctgcgcaggagcccaggggttggctgtgttccggccgcagagcaccgtctgcgtgaggagatcctggccaagttcctgcactggctgatgagtgtgtacgtcgtcgagctgctcaggtctttcttttatgtcacggagaccacgtttcaaaagaacaggctctttttctaccggaagagtgtctggagcaagttgcaaagcattggaatcagacagcacttgaagagggtgcagctgcgggagctgtcggaagcagaggtcaggcagcatcgggaagccaggcccgccctgctgacgtccagactccgcttcatccccaagcctgacgggctgcggccgattgtgaacatggactacgtcgtgggagccagaacgttccgcagagaaaagagggccgagcgtctcacctcgagggtgaaggcactgttcagcgtgctcaactacgagcgggcgcggcgccccggcctcctgggcgcctctgtgctgggcctggacgatatccacagggcctggcgcaccttcgtgctgcgtgtgcgggcccaggacccgccgcctgagctgtactttgtcaaggtggatgtgacgggcgcgtacgacaccatcccccaggacaggctcacggaggtcatcgccagcatcatcaaaccccagaacacgtactgcgtgcgtcggtatgccgtggtccagaaggccgcccatgggcacgtccgcaaggccttcaagagccacgtctctaccttgacagacctccagccgtacatgcgacagttcgtggctcacctgcaggagaccagcccgctgagggatgccgtcgtcatcgagcagagctcctccctgaatgaggccagcagtggcctcttcgacgtcttcctacgcttcatgtgccaccacgccgtgcgcatcaggggcaagtcctacgtccagtgccaggggatcccgcagggctccatcctctccacgctgctctgcagcctgtgctacggcgacatggagaacaagctgtttgcggggattcggcgggacgggctgctcctgcgtttggtggatgatttcttgttggtgacacctcacctcacccacgcgaaaaccttcctcaggaccctggtccgaggtgtccctgagtatggctgcgtggtgaacttgcggaagacagtggtgaacttccctgtagaagacgaggccctgggtggcacggcttttgttcagatgccggcccacggcctattcccctggtgcggcctgctgctggatacccggaccctggaggtgcagagcgactactccagctatgcccggacctccatcagagccagtctcaccttcaaccgcggcttcaaggctgggaggaacatgcgtcgcaaactctttggggtcttgcggctgaagtgtcacagcctgtttctggatttgcaggtgaacagcctccagacggtgtgcaccaacatctacaagatcctcctgctgcaggcgtacaggtttcacgcatgtgtgctgcagctcccatttcatcagcaagtttggaagaaccccacatttttcctgcgcgtcatctctgacacggcctccctctgctactccatcctgaaagccaagaacgcagggatgtcgctgggggccaagggcgccgccggccctctgccctccgaggccgtgcagtggctgtgccaccaagcattcctgctcaagctgactcgacaccgtgtcacctacgtgccactcctggggtcactcaggacagcccagacgcagctgagtcggaagctcccggggacgacgctgactgccctggaggccgcagccaacccggcactgccctcagacttcaagaccatcctggactga

SEQ ID NO: 6 - DNA, 3399 bp, Artificial sequence
  hoTERT long isoform
atgcctagagcacctagatgtagagctgtgcggagcctgctgcggagccactatagagaagttctgcccctggccaccttcgtgcgtagacttggacctcaaggatggcggctggtgcagagaggcgatcctgctgcttttagagccctggtggcccagtgtctcgtgtgcgttccatgggatgctagacctccaccagctgctcccagcttcagacaggtgtcctgcctgaaagaactggtggccagagtgctgcagcggctgtgtgaaaggggcgccaaaaatgtgctggccttcggctttgctctgctggatggtgctagaggcggacctcctgaggcctttacaacaagcgtgcggagctacctgcctaacaccgtgacagatgccctgagaggatctggcgcttggggactgctgctgagaagagtgggagatgacgtgctggtgcatctgctggctagatgcgccctgtttgtgctggtggctcctagctgtgcctaccaagtctgtggccctccactgtatcagctgggcgctgctacacaggctagaccacctccacatgccagcggacctagaagaaggctgggctgcgaaagagcctggaaccactctgttagagaagccggcgtgccactgggattgcctgcacctggtgcaagaagaagaggcggcagcgcctctagatctctgcctctgcctaagaggcctcggagaggtgctgctcctgagcctgagagaacacctgttggccaaggctcttgggcccatcctggcagaacaagaggccctagcgatagaggcttctgcgtggtgtctcctgccagacctgccgaggaagccacatctcttgaaggcgccctgagcggcacaagacactctcacccatctgtgggcagacagcaccatgccggacctccaagcacaagcagaccacctagaccttgggacaccccttgtcctccagtgtacgccgagacaaagcacttcctgtacagcagcggcgacaaagagcagctgaggcctagcttcctgctgtcctctctgaggccatctctgaccggtgctcggagactggtggaaaccatcttcctgggcagcagaccttggatgcccggcacacctagaaggctgcctagactgccacagcggtactggcaaatgaggcccctgttcctggaactgctgggcaatcacgctcagtgcccttatggcgtgctgctgaaaacccactgtcctctgagagccgccgtgacaccagcagctggcgtttgtgccagagagaagcctcaaggctctgtggctgcccctgaggaagaggacacagatcctagacgactggtgcagctcctgcggcagcattctagtccatggcaggtctacggattcgtgcgggcctgtctgagaaggcttgttcctcctggactgtggggctccagacacaacgagcggcggtttctgcggaacaccaagaagttcatcagcctgggaaagcacgccaagctgagcctgcaagagctgacctggaagatgagcgtgcgggattgtgcatggctgagaaggtccccaggcgtgggatgtgttcctgccgctgaacacagactgcgggaagagatcctggccaagttcctgcactggctgatgtccgtgtacgtggtcgaactgcttcggagcttcttctacgtgaccgagacaaccttccagaagaaccggctgttcttctaccggaagtccgtgtggtccaagctgcagagcatcggcattcggcagcacctgaagagagtgcagctgagagagctgagcgaggctgaagtccggcagcacagagaagctagaccagctctgctgaccagcaggctgagattcatccccaagcctgatggcctgcggcctatcgtgaacatggactatgttgtgggcgccagaacctttcggagagagaagagagccgagcggctgacctctagagtgaaggccctgttcagcgtgctgaactacgagagagccagaaggcctggactgctcggagcctctgttctgggcctcgacgatatccacagagcttggcggacctttgtgctgagagtcagagcccaggatcctccacctgagctgtacttcgtgaaggtggacgtgaccggcgcctacgacacaatccctcaggacagactgaccgaagtgatcgccagcatcatcaagccccagaacacctactgtgtgcggagatacgccgtggtgcagaaagccgctcatggacatgtgcgcaaggccttcaagtcccacgtgtccacactgaccgacctgcagccttacatgagacagttcgtggcccatctgcaagagacaagccctctgagggatgccgtggtcatcgaacagagcagcagcctgaatgaggccagctccggcctgtttgacgtgttcctcagattcatgtgccaccacgccgtgcggatcagaggcaagagctatgtgcagtgccagggcattccacagggcagcatcctgagcacactgctgtgcagcctgtgctacggcgacatggaaaacaagctgttcgccggcatcagacgcgacggcctgcttctgagactggtcgacgatttcctgctcgtgacccctcacctgacacacgccaagacctttctgagaacactcgtgcggggcgtgccagagtatggctgtgtggtcaacctgagaaagaccgtggtcaacttccccgtcgaggatgaagcccttggcggcacagctttcgtgcagatgcctgctcacggactgttcccttggtgcggactgctcctggacaccagaacactggaagtgcagagcgactacagcagctacgcccggacatctatcagagccagcctgaccttcaaccggggctttaaggccggcagaaacatgcggagaaagctgtttggagtgctgcggctgaagtgccactctttgtttctggacctgcaagtgaacagcctgcagaccgtgtgcaccaacatctacaagattctgctgctgcaagcctaccggttccacgcctgtgttctgcagctgcccttccaccagcaagtgtggaagaaccctacattcttcctgcgcgtgatcagcgacaccgccagcctgtgttactccatcctgaaggccaagaacgccggcatgtctctgggagctaaaggcgctgctggacctctgccttctgaagcagtgcagtggctctgccaccaggcctttctgctgaagctgaccagacacagagtgacctacgtgcccctgctgggctcactgagaacagctcagacacagctgagcagaaagctgcctggcacaaccctgacagccctggaagctgcagcaaaccctgctctgcccagcgacttcaagaccatcctggattga

SEQ ID NO: 7 - protein, 1132 aa, Homo sapiens
  hTERT long isoform protein
MPRAPRCRAVRSLLRSHYREVLPLATFVRRLGPQGWRLVQRGDPAAFRALVAQCLVCVPWDARPPPAAPSFRQVSCLKELVARVLQRLCERGAKNVLAFGFALLDGARGGPPEAFTTSVRSYLPNTVTDALRGSGAWGLLLRRVGDDVLVHLLARCALFVLVAPSCAYQVCGPPLYQLGAATQARPPPHASGPRRRLGCERAWNHSVREAGVPLGLPAPGARRRGGSASRSLPLPKRPRRGAAPEPERTPVGQGSWAHPGRTRGPSDRGFCVVSPARPAEEATSLEGALSGTRHSHPSVGRQHHAGPPSTSRPPRPWDTPCPPVYAETKHFLYSSGDKEQLRPSFLLSSLRPSLTGARRLVETIFLGSRPWMPGTPRRLPRLPQRYWQMRPLFLELLGNHAQCPYGVLLKTHCPLRAAVTPAAGVCAREKPQGSVAAPEEEDTDPRRLVQLLRQHSSPWQVYGFVRACLRRLVPPGLWGSRHNERRFLRNTKKFISLGKHAKLSLQELTWKMSVRDCAWLRRSPGVGCVPAAEHRLREEILAKFLHWLMSVYVVELLRSFFYVTETTFQKNRLFFYRKSVWSKLQSIGIRQHLKRVQLRELSEAEVRQHREARPALLTSRLRFIPKPDGLRPIVNMDYVVGARTFRREKRAERLTSRVKALFSVLNYERARRPGLLGASVLGLDDIHRAWRTFVLRVRAQDPPPELYFVKVDVTGAYDTIPQDRLTEVIASIIKPQNTYCVRRYAVVQKAAHGHVRKAFKSHVSTLTDLQPYMRQFVAHLQETSPLRDAVVIEQSSSLNEASSGLFDVFLRFMCHHAVRIRGKSYVQCQGIPQGSILSTLLCSLCYGDMENKLFAGIRRDGLLLRLVDDFLLVTPHLTHAKTFLRTLVRGVPEYGCVVNLRKTVVNFPVEDEALGGTAFVQMPAHGLFPWCGLLLDTRTLEVQSDYSSYARTSIRASLTFNRGFKAGRNMRRKLFGVLRLKCHSLFLDLQVNSLQTVCTNIYKILLLQAYRFHACVLQLPFHQQVWKNPTFFLRVISDTASLCYSILKAKNAGMSLGAKGAAGPLPSEAVQWLCHQAFLLKLTRHRVTYVPLLGSLRTAQTQLSRKLPGTTLTALEAAANPALPSDFKTILD

SEQ ID NO: 8 - DNA, 3210 bp, Homo sapiens
  hTERT short isoform
atgccgcgcgctccccgctgccgagccgtgcgctccctgctgcgcagccactaccgcgaggtgctgccgctggccacgttcgtgcggcgcctggggccccagggctggcggctggtgcagcgcggggacccggcggctttccgcgcgctggtggcccagtgcctggtgtgcgtgccctgggacgcacggccgccccccgccgccccctccttccgccaggtgtcctgcctgaaggagctggtggcccgagtgctgcagaggctgtgcgagcgcggcgcgaagaacgtgctggccttcggcttcgcgctgctggacggggcccgcgggggcccccccgaggccttcaccaccagcgtgcgcagctacctgcccaacacggtgaccgacgcactgcgggggagcggggcgtgggggctgctgctgcgccgcgtgggcgacgacgtgctggttcacctgctggcacgctgcgcgctctttgtgctggtggctcccagctgcgcctaccaggtgtgcgggccgccgctgtaccagctcggcgctgccactcaggcccggcccccgccacacgctagtggaccccgaaggcgtctgggatgcgaacgggcctggaaccatagcgtcagggaggccggggtccccctgggcctgccagccccgggtgcgaggaggcgcgggggcagtgccagccgaagtctgccgttgcccaagaggcccaggcgtggcgctgcccctgagccggagcggacgcccgttgggcaggggtcctgggcccacccgggcaggacgcgtggaccgagtgaccgtggtttctgtgtggtgtcacctgccagacccgccgaagaagccacctctttggagggtgcgctctctggcacgcgccactcccacccatccgtgggccgccagcaccacgcgggccccccatccacatcgcggccaccacgtccctgggacacgccttgtcccccggtgtacgccgagaccaagcacttcctctactcctcaggcgacaaggagcagctgcggccctccttcctactcagctctctgaggcccagcctgactggcgctcggaggctcgtggagaccatctttctgggttccaggccctggatgccagggactccccgcaggttgccccgcctgccccagcgctactggcaaatgcggcccctgtttctggagctgcttgggaaccacgcgcagtgcccctacggggtgctcctcaagacgcactgcccgctgcgagctgcggtcaccccagcagccggtgtctgtgcccgggagaagccccagggctctgtggcggcccccgaggaggaggacacagacccccgtcgcctggtgcagctgctccgccagcacagcagcccctggcaggtgtacggcttcgtgcgggcctgcctgcgccggctggtgcccccaggcctctggggctccaggcacaacgaacgccgcttcctcaggaacaccaagaagttcatctccctggggaagcatgccaagctctcgctgcaggagctgacgtggaagatgagcgtgcgggactgcgcttggctgcgcaggagcccaggggttggctgtgttccggccgcagagcaccgtctgcgtgaggagatcctggccaagttcctgcactggctgatgagtgtgtacgtcgtcgagctgctcaggtctttcttttatgtcacggagaccacgtttcaaaagaacaggctctttttctaccggaagagtgtctggagcaagttgcaaagcattggaatcagacagcacttgaagagggtgcagctgcgggagctgtcggaagcagaggtcaggcagcatcgggaagccaggcccgccctgctgacgtccagactccgcttcatccccaagcctgacgggctgcggccgattgtgaacatggactacgtcgtgggagccagaacgttccgcagagaaaagagggccgagcgtctcacctcgagggtgaaggcactgttcagcgtgctcaactacgagcgggcgcggcgccccggcctcctgggcgcctctgtgctgggcctggacgatatccacagggcctggcgcaccttcgtgctgcgtgtgcgggcccaggacccgccgcctgagctgtactttgtcaaggtggatgtgacgggcgcgtacgacaccatcccccaggacaggctcacggaggtcatcgccagcatcatcaaaccccagaacacgtactgcgtgcgtcggtatgccgtggtccagaaggccgcccatgggcacgtccgcaaggccttcaagagccacgtctctaccttgacagacctccagccgtacatgcgacagttcgtggctcacctgcaggagaccagcccgctgagggatgccgtcgtcatcgagcagagctcctccctgaatgaggccagcagtggcctcttcgacgtcttcctacgcttcatgtgccaccacgccgtgcgcatcaggggcaagtcctacgtccagtgccaggggatcccgcagggctccatcctctccacgctgctctgcagcctgtgctacggcgacatggagaacaagctgtttgcggggattcggcgggacgggctgctcctgcgtttggtggatgatttcttgttggtgacacctcacctcacccacgcgaaaaccttcctcagctatgcccggacctccatcagagccagtctcaccttcaaccgcggcttcaaggctgggaggaacatgcgtcgcaaactctttggggtcttgcggctgaagtgtcacagcctgtttctggatttgcaggtgaacagcctccagacggtgtgcaccaacatctacaagatcctcctgctgcaggcgtacaggtttcacgcatgtgtgctgcagctcccatttcatcagcaagtttggaagaaccccacatttttcctgcgcgtcatctctgacacggcctccctctgctactccatcctgaaagccaagaacgcagggatgtcgctgggggccaagggcgccgccggccctctgccctccgaggccgtgcagtggctgtgccaccaagcattcctgctcaagctgactcgacaccgtgtcacctacgtgccactcctggggtcactcaggacagcccagacgcagctgagtcggaagctcccggggacgacgctgactgccctggaggccgcagccaacccggcactgccctcagacttcaagaccatcctggactga

SEQ ID NO: 9 - DNA, 3210 bp, Artificial sequence
  hoTERT short isoform
atgcctcgggctcctagatgtagagccgtcagaagcctgctgcggagccactatagagaggtgctgcctctggccaccttcgtgcgtagacttggacctcaaggatggcggctggtgcagagaggcgatcctgctgcttttagagccctggtggcccagtgtctcgtgtgcgttccatgggatgctagacctccaccagctgctcccagcttcagacaggtgtcctgcctgaaagaactggtggccagggtgctgcagagactgtgtgaaaggggcgccaagaacgtgctggcctttggatttgctctgctggatggcgctagaggcggacctcctgaggcctttacaacaagcgtgcggagctacctgcctaacaccgtgacagatgccctgagaggatctggcgcttggggactgctgctgagaagagtgggagatgacgtgctggtgcatctgctggccagatgcgctctgtttgtgctggtggctcctagctgcgcctaccaagtttgtggccctccactgtatcagctgggcgctgctacacaggctagaccacctccacatgccagcggacctagaagaaggctgggctgcgaaagagcctggaaccactctgttagagaagccggcgtgccactgggattgcctgcaccaggtgcaagaagaagaggcggcagcgcctctagatctctgcctctgcctaagaggcctagaagaggggctgcccctgagcctgagagaacacctgttggccaaggctcttgggcccatcctggcagaacaagaggccctagcgatagaggcttctgcgtggtgtctcctgccagacctgccgaggaagccacatctcttgaaggcgccctgagcggcacaagacactctcacccatctgtgggcagacagcaccatgccggacctccaagcacaagcagaccacctagaccttgggacaccccttgtcctccagtgtacgccgagacaaagcacttcctgtacagcagcggcgacaaagagcagctgaggcctagcttcctgctgtcctctctgaggccatctctgaccggtgctcggagactggtggaaaccatcttcctgggcagcagaccttggatgcccggcacacctagaaggctgcctagactgccacagcggtactggcaaatgaggcccctgttcctggaactgctgggcaatcacgctcagtgcccttatggcgtgctgctgaaaacccactgtcctctgagagccgccgtgacaccagcagctggcgtttgtgccagagagaagcctcaaggctctgtggccgctcctgaggaagaggacacagatcctagacgactggtgcagctcctgagacagcacagctctccatggcaggtctacggatttgtgcgggcctgtctgagaaggctcgttcctcctggactgtggggctccagacacaacgagcggcggtttctgcggaacaccaagaagttcatcagcctgggaaagcacgccaagctgagcctgcaagagctgacctggaagatgagcgtgcgggattgtgcatggctgagaaggtccccaggcgtgggatgtgttcctgccgctgaacacagactgcgggaagagatcctggccaagttcctgcactggctgatgtccgtgtacgtggtcgaactgcttcggagcttcttctacgtgaccgagacaaccttccagaagaaccggctgttcttctaccggaagtccgtgtggtccaagctgcagagcatcggcatccggcagcatctgaagagagtgcagctgagagagctgagcgaagccgaagtgcggcagcacagagaagctagaccagctctgctgaccagcaggctgagattcatccccaagcctgatggcctgcggcctatcgtgaacatggactatgttgtgggcgccagaacctttcggagagagaagagagccgagcggctgacctctagagtgaaggccctgttcagcgtgctgaactacgagagagccagaaggccaggactgctgggagcctctgttctgggcctcgacgatatccacagagcttggcggacctttgtgctgagagtgcgagcccaagatcctccacctgagctgtacttcgtgaaggtggacgtgaccggcgcctacgacacaatccctcaggacagactgaccgaagtgatcgccagcatcatcaagccccagaacacctactgtgtgcggagatacgccgtggtgcagaaagccgctcatggacatgtgcgcaaggccttcaagtcccacgtgtccacactgaccgacctgcagccttacatgagacagttcgtggcccatctgcaagagacaagccctctgagggatgccgtggtcatcgaacagagcagcagcctgaatgaggccagctccggcctgtttgacgtgttcctcagattcatgtgccaccacgccgtgcggatcagaggcaagagctatgtgcagtgccagggcattcctcagggcagcatcctgagcacactgctgtgcagcctgtgctacggcgacatggaaaacaagctgttcgccggcatcagacgcgacggcctgcttctgagactggtcgacgatttcctgctcgtgacccctcacctgacacacgccaagacctttctgagctacgcccggacctctatcagagccagcctgaccttcaaccggggctttaaggccggcagaaacatgcggagaaagctgtttggagtgctgcggctgaagtgccactctttgtttctggacctgcaagtgaacagcctgcagaccgtgtgcaccaacatctacaagattctgctgctgcaagcctaccggttccacgcctgtgttctgcagctgccctttcaccagcaagtgtggaagaaccctacattcttcctgcgcgtgatcagcgacaccgccagcctgtgttactccatcctgaaggccaaaaacgccggcatgagcctgggagctaaaggcgctgctggacctctgccttctgaagcagtgcagtggctgtgtcaccaggcctttctgctgaagctgacccggcacagagtgacatatgtgcctctgctgggctccctgagaaccgctcaaacacagctgagcagaaagctgcctggcacaaccctgacagccctggaagctgcagcaaaccctgctctgcccagcgacttcaagaccatcctggattga

SEQ ID NO: 10 - protein, 1069 aa, Homo sapiens
  hTERT short isoform protein
MPRAPRCRAVRSLLRSHYREVLPLATFVRRLGPQGWRLVQRGDPAAFRALVAQCLVCVPWDARPPPAAPSFRQVSCLKELVARVLQRLCERGAKNVLAFGFALLDGARGGPPEAFTTSVRSYLPNTVTDALRGSGAWGLLLRRVGDDVLVHLLARCALFVLVAPSCAYQVCGPPLYQLGAATQARPPPHASGPRRRLGCERAWNHSVREAGVPLGLPAPGARRRGGSASRSLPLPKRPRRGAAPEPERTPVGQGSWAHPGRTRGPSDRGFCVVSPARPAEEATSLEGALSGTRHSHPSVGRQHHAGPPSTSRPPRPWDTPCPPVYAETKHFLYSSGDKEQLRPSFLLSSLRPSLTGARRLVETIFLGSRPWMPGTPRRLPRLPQRYWQMRPLFLELLGNHAQCPYGVLLKTHCPLRAAVTPAAGVCAREKPQGSVAAPEEEDTDPRRLVQLLRQHSSPWQVYGFVRACLRRLVPPGLWGSRHNERRFLRNTKKFISLGKHAKLSLQELTWKMSVRDCAWLRRSPGVGCVPAAEHRLREEILAKFLHWLMSVYVVELLRSFFYVTETTFQKNRLFFYRKSVWSKLQSIGIRQHLKRVQLRELSEAEVRQHREARPALLTSRLRFIPKPDGLRPIVNMDYVVGARTFRREKRAERLTSRVKALFSVLNYERARRPGLLGASVLGLDDIHRAWRTFVLRVRAQDPPPELYFVKVDVTGAYDTIPQDRLTEVIASIIKPQNTYCVRRYAVVQKAAHGHVRKAFKSHVSTLTDLQPYMRQFVAHLQETSPLRDAVVIEQSSSLNEASSGLFDVFLRFMCHHAVRIRGKSYVQCQGIPQGSILSTLLCSLCYGDMENKLFAGIRRDGLLLRLVDDFLLVTPHLTHAKTFLSYARTSIRASLTFNRGFKAGRNMRRKLFGVLRLKCHSLFLDLQVNSLQTVCTNIYKILLLQAYRFHACVLQLPFHQQVWKNPTFFLRVISDTASLCYSILKAKNAGMSLGAKGAAGPLPSEAVQWLCHQAFLLKLTRHRVTYVPLLGSLRTAQTQLSRKLPGTTLTALEAAANPALPSDFKTILD

SEQ ID NO: 11 - DNA, 1597 bp, Artificial sequence
  SpB promoter full length
aataacaagcacgtttcagttccaccttcctgaggttctaccaaggtcactcagttcccagtctttggttactcatttttacacagtcttggtggactcccatgatggcagctgtgtttgttgtactgacaaggacttgaggccaacagaaactacataaatccttgggtaaccttgagtgtggcattagccaccttgtatctaattctttttttttttttttttttgagacagagtgttacctggccaacatggtgtcaggagactgcccatcccagggaccaggagccaggacaccctcagctcagtcacatgtttaatggccacatgtttaatggcctcacactcccattccagagtgcagcggtgcaatcatggctcactgcagccgcgacctggtgggctcaagcgatcctcctgccccagctttctgagtagctgggaccagagacatgcaccaccacacaaggttaattttttaatttttttgtagttatggagtcttactatattggccaggctggtctcaaactccagggctcaaaggatcctccctcctcggcctcccaaagtgccaggattacaggagtgagccaccacacccagccccatctcttttcatcatggtactaattcctgcccgtccacccacaaaagcactgtagtgcttcccgagtatagaggcctgtgagcctccactagggagagggctcctgcagagatcagataaattgatcacaatggctggggtggtggcaatgtgctaatgctctctttcttccactcaagatatcctctgtctccctcagcctgtgagctttttctccagtgtgctctgccagtgggggccctgcctgagagcccctgcagctgcagaggacagtttctttctgctgaaccatcgcagctatgccccagcccctaccctggaggggtccccaggggccatgggcagcacctcctgtatagggctgtctgggagccactccagggccacagaaatcttgtctctgactcagggtattttgttttctgttttgtgtaaatgctcttctgactaatgcaaaccatgtgtccatagaaccagaagatttttccaggggaaaaggtaaggaggtggtgagagtgtcctgggtctgcccttccagggcttgccctgggttaagagccaggcaggaagctctcaagagcattgctcaagagtagagggggcctgggaggcccagggaggggatgggaggggaacacccaggctgcccccaaccagatgccctccaccctcctcaacctccctcccacggcctggagaggtgggaccaggtatggaggcttgagagcccctggttggaggaagccacaagtccaggaacatgggagtctgggcagggggcaaaggaggcaggaacaggccatcagccaggacaggtggtaaggcaggcaggagtgttcctgctgggaaaaggtgggatcaagcacctggagggctcttcagagcaaagacaaacactgaggtcgctgccactcctacagagcccccacgccccgcccagctataaggggccatgcaccaagcagggtacccaggctgcagaggtgc

SEQ ID NO: 12 - DNA, 632 bp, Artificial sequence
  SpB promoter shortened
atagggctgtctgggagccactccagggccacagaaatcttgtctctgactcagggtattttgttttctgttttgtgtaaatgctcttctgactaatgcaaaccatgtgtccatagaaccagaagatttttccaggggaaaaggtaaggaggtggtgagagtgtcctgggtctgcccttccagggcttgccctgggttaagagccaggcaggaagctctcaagagcattgctcaagagtagagggggcctgggaggcccagggaggggatgggaggggaacacccaggctgcccccaaccagatgccctccaccctcctcaacctccctcccacggcctggagaggtgggaccaggtatggaggcttgagagcccctggttggaggaagccacaagtccaggaacatgggagtctgggcagggggcaaaggaggcaggaacaggccatcagccaggacaggtggtaaggcaggcaggagtgttcctgctgggaaaaggtgggatcaagcacctggagggctcttcagagcaaagacaaacactgaggtcgctgccactcctacagagcccccacgccccgcccagctataaggggccatgcaccaagcagggtacccaggctgcagaggtgc

SEQ ID NO: 13 - DNA, 296 bp, Artificial sequence
  MLC2v promoter shortened
gttaacgtttaaacttagacaatggcaggacccagagcacagagcatcgttcccaggccaggccccagccactgtctctttaaccttgaaggcatttttgggtctcacgtgtccacccaggcgggtgtcggactttgaacggctcttacttcagaagaacggcatggggtgggggggcttaggtggcctctgcctcacctacaactgccaaaagtggtcatggggttatttttaaccccagggaagaggtatttattgttccacagcaggggccggccagcaggctccttgaattc

SEQ ID NO: 14 - DNA, 380 bp, Artificial sequence
  CMV enhancer
gacattgattattgactagttattaatagtaatcaattacggggtcattagttcatagcccatatatggagttccgcgttacataacttacggtaaatggcccgcctggctgaccgcccaacgacccccgcccattgacgtcaataatgacgtatgttcccatagtaacgccaatagggactttccattgacgtcaatgggtggactatttacggtaaactgcccacttggcagtacatcaagtgtatcatatgccaagtacgccccctattgacgtcaatgacggtaaatggcccgcctggcattatgcccagtacatgaccttatgggactttcctacttggcagtacatctacgtattagtcatcgctattaccatg

SEQ ID NO: 15 - DNA, 676 bp, Artificial sequence
  CMVenh-MLC2v promoter
gacattgattattgactagttattaatagtaatcaattacggggtcattagttcatagcccatatatggagttccgcgttacataacttacggtaaatggcccgcctggctgaccgcccaacgacccccgcccattgacgtcaataatgacgtatgttcccatagtaacgccaatagggactttccattgacgtcaatgggtggactatttacggtaaactgcccacttggcagtacatcaagtgtatcatatgccaagtacgccccctattgacgtcaatgacggtaaatggcccgcctggcattatgcccagtacatgaccttatgggactttcctacttggcagtacatctacgtattagtcatcgctattaccatggttaacgtttaaacttagacaatggcaggacccagagcacagagcatcgttcccaggccaggccccagccactgtctctttaaccttgaaggcatttttgggtctcacgtgtccacccaggcgggtgtcggactttgaacggctcttacttcagaagaacggcatggggtgggggggcttaggtggcctctgcctcacctacaactgccaaaagtggtcatggggttatttttaaccccagggaagaggtatttattgttccacagcaggggccggccagcaggctccttgaattc

SEQ ID NO: 16 - DNA, 544 bp, Artificial sequence
  TNT promoter shortened
ctcagtccattaggagccagtagcctggaagatgtctttacccccagcatcagttcaagtggagcagcacataactcttgccctctgccttccaagattctggtgctgagacttatggagtgtcttggaggttgccttctgccccccaaccctgctcccagctggccctcccaggcctgggttgctggcctctgctttatcaggattctcaagagggacagctggtttatgttgcatgactgttccctgcatatctgctctggttttaaatagcttatctgagcagctggaggaccacatgggcttatatggcgtggggtacatgttcctgtagccttgtccctggcacctgccaaaatagcagccaacaccccccacccccaccgccatccccctgccccacccgtcccctgtcgcacattcctccctccgcagggctggctcaccaggccccagcccacatgcctgcttaaagccctctccatcctctgcctcacccagtccccgctgagactgagcagacgcctccaggatctgtcggcag

SEQ ID NO: 17 - RNA, 7 nt, Artificial sequence
  kozak sequence
accaugg

SEQ ID NO: 18 - DNA, 225 bp, Artificial sequence
  BGH polyA
ctgtgccttctagttgccagccatctgttgtttgcccctcccccgtgccttccttgaccctggaaggtgccactcccactgtcctttcctaataaaatgaggaaattgcatcgcattgtctgagtaggtgtcattctattctggggggtggggtggggcaggacagcaagggggaggattgggaagacaatagcaggcatgctggggatgcggtgggctctatgg

SEQ ID NO: 19 - DNA, 141 bp, Artificial sequence
  5' ITR AAV2
cctgcaggcagctgcgcgctcgctcgctcactgaggccgcccgggcaaagcccgggcgtcgggcgacctttggtcgcccggcctcagtgagcgagcgagcgcgcagagagggagtggccaactccatcactaggggttcct

SEQ ID NO: 20 - DNA, 141 bp, Artificial sequence
  3' ITR AAV2
aggaacccctagtgatggagttggccactccctctctgcgcgctcgctcgctcactgaggccgggcgaccaaaggtcgcccgacgcccgggctttgcccgggcggcctcagtgagcgagcgagcgcgcagctgcctgcagg

SEQ ID NO: 21 - DNA, 4638 bp, Artificial sequence
  AAV-SpB-moTERT recombinant adeno-associated virus genome
cctgcaggcagctgcgcgctcgctcgctcactgaggccgcccgggcaaagcccgggcgtcgggcgacctttggtcgcccggcctcagtgagcgagcgagcgcgcagagagggagtggccaactccatcactaggggttcctgcggccgcgatatcatagggctgtctgggagccactccagggccacagaaatcttgtctctgactcagggtattttgttttctgttttgtgtaaatgctcttctgactaatgcaaaccatgtgtccatagaaccagaagatttttccaggggaaaaggtaaggaggtggtgagagtgtcctgggtctgcccttccagggcttgccctgggttaagagccaggcaggaagctctcaagagcattgctcaagagtagagggggcctgggaggcccagggaggggatgggaggggaacacccaggctgcccccaaccagatgccctccaccctcctcaacctccctcccacggcctggagaggtgggaccaggtatggaggcttgagagcccctggttggaggaagccacaagtccaggaacatgggagtctgggcagggggcaaaggaggcaggaacaggccatcagccaggacaggtggtaaggcaggcaggagtgttcctgctgggaaaaggtgggatcaagcacctggagggctcttcagagcaaagacaaacactgaggtcgctgccactcctacagagcccccacgccccgcccagctataaggggccatgcaccaagcagggtacccaggctgcagaggtgcgaattcatttaaattctagatcgctagcacgcgtgccaccatgacaagagcccctagatgtcctgccgtcagaagcctgctgagaagcagatacagagaagtgtggcccctggccaccttcgtcagaaggcttggacctgaaggcagacggctggttcaacctggcgaccccaagatctacagaaccctggtggctcagtgcctcgtgtgtatgcactggggatctcagccacctcctgccgatctgagctttcaccaggtgtccagcctgaaagaactggtggccagagtggtgcagagactgtgcgagagaaacgagaggaacgtgctggccttcggcttcgagctgctgaatgaagctagaggcggccctcctatggccttcacatctagcgtgcggagctacctgcctaacaccgtgatcgagacactgagagtgtccggcgcttggatgctgctgctgagcagagtgggagatgacctgctggtgtacctgctggctcactgtgccctctatctgctggtgcctcctagctgcgcttaccaagtgtgcggaagccctctgtaccagatctgtgccaccaccgacatctggcctagcgtgtccgcttcctacagacccacaagacccgtgggcagaaactttaccaacctgagattcctgcagcagatcaagagcagctccaggcaagaggcccctaagcctcttgctctgcctagcagaggcaccaagagacacctgagcctgaccagcacaagcgtgccctctgccaagaaagccagatgctaccccgtgcctagagtggaagagggcccacatagacaggtgctgcctacacctagcggcaagagctgggttccatctcctgctagaagccctgaggtgccaacagccgagaaggacctgagcagcaagggcaaagtgtccgacctgtctctgagcggcagcgtgtgttgcaagcacaagcctagcagcaccagcctgctgtccccacctagacagaacgctttccagctgaggccctttatcgagacaagacacttcctgtacagcagaggcgacggccaagagagactgaaccctagcttcctgctgtctaacctgcagcctaacctgaccggcgctagaaggctggtggaaatcatcttcctgggcagcagacccagaaccagcggacctctgtgtagaacccacagactgagcagacggtactggcagatgaggcccctgttccagcagctcctggtcaaccatgccgagtgtcagtatgtgcggctgctgaggtcccactgcagattcagaaccgccaaccagcaagtgacagacgccctgaacacaagccctccacacctgatggatctgctgagactgcacagcagcccctggcaggtctacggctttctgagagcctgtctgtgcaaggtggtgtccgcatctctgtggggcaccagacacaacgagagaagattcttcaagaacctgaagaagttcatcagcctggggaagtacggcaagctgtccctgcaagaactgatgtggaagatgaaggtcgaggactgccactggctgaggtctagccctggcaaggatagagtgcctgccgctgagcacaggctgagagagagaatcctggccacattcctgttctggctgatggacacctacgtggtgcagctgctgcggagcttcttctacatcaccgagagcaccttccagaagaaccggctgttcttctaccgcaagagcgtgtggtccaagctgcagagcatcggcgtcagacagcacctggaaagagtgcgcctgagagagctgagccaagaggaagtgcggcaccaccaggatacctggctggccatgcctatctgcagactgagattcatccccaagcctaacggcctgaggcctatcgtgaacatgagctacagcatgggcactagagccctgggcagaagaaagcaggcccagcacttcacccagaggctgaaaaccctgttctccatgctgaactacgagcggacaaagcaccctcatctgatgggctcctctgtgctgggcatgaacgacatctacaggacctggcgggccttcgtgctgagagtcagagcactggaccagacacctagaatgtacttcgtgaaggccgacgtgacaggcgcctacgatgctatccctcagggcaaactggtggaagtggtggccaacatgatcaggcacagcgagtccacctactgcatcagacagtacgccgtcgtgcggagagactctcagggacaagtgcacaagagcttccgcagacaagtgaccacactgagcgatctgcagccctacatgggccagtttctgaagcacctccaggacagcgacgccagcgctctgagaaactctgtggtcatcgagcagtccatctccatgaacgagtccagctccagcctgttcgacttcttcctgcacttcctgcggcacagcgtggtcaagatcggcgacagatgttacacccagtgccagggcatcccacagggaagcagtctgagcacactgctgtgctccctgtgtttcggcgacatggaaaacaagctgttcgccgaagtgcagcgcgacggactgctcctgagatttgtggacgacttcctgctcgtgacccctcacctggatcaggctaagaccttcctgagcaccctggtgcatggcgtgccagagtacggctgcatgatcaacctgcagaaaaccgtggtcaacttccccgtggaacctggcactcttggaggcgctgctccttatcagctgcccgctcattgtctgttcccttggtgcggactgctgctggacacacagaccctggaagtgttctgcgactacagcggctacgcccagaccagcatcaagaccagcctgaccttccagtccgtgttcaaggccggcaagaccatgaggaacaagctgctgagtgtgctgaggctgaagtgccacggcctgtttctggacctgcaagtgaacagcctgcagaccgtgtgcatcaatatctacaagatctttctgctgcaagcctaccggttccacgcctgtgtgattcagctgcctttcgaccagagagtgcggaagaatctgacattctttctgggcatcatcagcagccaggccagctgctgttacgccatcctgaaagtgaagaaccccggcatgaccctgaaggcctctggcagctttccacctgaagctgcccattggctgtgctaccaggctttcctgctgaaactggctgcccacagcgtgatctacaagtgcctgctgggcccactgagaacagcccagaaactgctgtgtcggaagctgcctgaagccacaatgacaatcctgaaggctgccgccgatccagctctgagcaccgacttccagaccatcctggactgagaattcggatccgattcgagcatttaaatacgtggagctcgctgatcagcctcgactgtgccttctagttgccagccatctgttgtttgcccctcccccgtgccttccttgaccctggaaggtgccactcccactgtcctttcctaataaaatgaggaaattgcatcgcattgtctgagtaggtgtcattctattctggggggtggggtggggcaggacagcaagggggaggattgggaagacaatagcaggcatgctggggatgcggtgggctctatggccacgtggatatcgcggccgcaggaacccctagtgatggagttggccactccctctctgcgcgctcgctcgctcactgaggccgggcgaccaaaggtcgcccgacgcccgggctttgcccgggcggcctcagtgagcgagcgagcgcgcagctgcctgcagg

SEQ ID NO: 22 - DNA, 4676 bp, Artificial sequence
  AAV9-CMVenh-MLC2v-moTERT
cctgcaggcagctgcgcgctcgctcgctcactgaggccgcccgggcaaagcccgggcgtcgggcgacctttggtcgcccggcctcagtgagcgagcgagcgcgcagagagggagtggccaactccatcactaggggttcctgcggccgcgatatcgacattgattattgactagttattaatagtaatcaattacggggtcattagttcatagcccatatatggagttccgcgttacataacttacggtaaatggcccgcctggctgaccgcccaacgacccccgcccattgacgtcaataatgacgtatgttcccatagtaacgccaatagggactttccattgacgtcaatgggtggactatttacggtaaactgcccacttggcagtacatcaagtgtatcatatgccaagtacgccccctattgacgtcaatgacggtaaatggcccgcctggcattatgcccagtacatgaccttatgggactttcctacttggcagtacatctacgtattagtcatcgctattaccatggttaacgtttaaacttagacaatggcaggacccagagcacagagcatcgttcccaggccaggccccagccactgtctctttaaccttgaaggcatttttgggtctcacgtgtccacccaggcgggtgtcggactttgaacggctcttacttcagaagaacggcatggggtgggggggcttaggtggcctctgcctcacctacaactgccaaaagtggtcatggggttatttttaaccccagggaagaggtatttattgttccacagcaggggccggccagcaggctccttgaattcatttaaattctagatcgctagcacgcgtgccaccatgacaagagcccctagatgtcctgccgtcagaagcctgctgagaagcagatacagagaagtgtggcccctggccaccttcgtcagaaggcttggacctgaaggcagacggctggttcaacctggcgaccccaagatctacagaaccctggtggctcagtgcctcgtgtgtatgcactggggatctcagccacctcctgccgatctgagctttcaccaggtgtccagcctgaaagaactggtggccagagtggtgcagagactgtgcgagagaaacgagaggaacgtgctggccttcggcttcgagctgctgaatgaagctagaggcggccctcctatggccttcacatctagcgtgcggagctacctgcctaacaccgtgatcgagacactgagagtgtccggcgcttggatgctgctgctgagcagagtgggagatgacctgctggtgtacctgctggctcactgtgccctctatctgctggtgcctcctagctgcgcttaccaagtgtgcggaagccctctgtaccagatctgtgccaccaccgacatctggcctagcgtgtccgcttcctacagacccacaagacccgtgggcagaaactttaccaacctgagattcctgcagcagatcaagagcagctccaggcaagaggcccctaagcctcttgctctgcctagcagaggcaccaagagacacctgagcctgaccagcacaagcgtgccctctgccaagaaagccagatgctaccccgtgcctagagtggaagagggcccacatagacaggtgctgcctacacctagcggcaagagctgggttccatctcctgctagaagccctgaggtgccaacagccgagaaggacctgagcagcaagggcaaagtgtccgacctgtctctgagcggcagcgtgtgttgcaagcacaagcctagcagcaccagcctgctgtccccacctagacagaacgctttccagctgaggccctttatcgagacaagacacttcctgtacagcagaggcgacggccaagagagactgaaccctagcttcctgctgtctaacctgcagcctaacctgaccggcgctagaaggctggtggaaatcatcttcctgggcagcagacccagaaccagcggacctctgtgtagaacccacagactgagcagacggtactggcagatgaggcccctgttccagcagctcctggtcaaccatgccgagtgtcagtatgtgcggctgctgaggtcccactgcagattcagaaccgccaaccagcaagtgacagacgccctgaacacaagccctccacacctgatggatctgctgagactgcacagcagcccctggcaggtctacggctttctgagagcctgtctgtgcaaggtggtgtccgcatctctgtggggcaccagacacaacgagagaagattcttcaagaacctgaagaagttcatcagcctggggaagtacggcaagctgtccctgcaagaactgatgtggaagatgaaggtcgaggactgccactggctgaggtctagccctggcaaggatagagtgcctgccgctgagcacaggctgagagagagaatcctggccacattcctgttctggctgatggacacctacgtggtgcagctgctgcggagcttcttctacatcaccgagagcaccttccagaagaaccggctgttcttctaccgcaagagcgtgtggtccaagctgcagagcatcggcgtcagacagcacctggaaagagtgcgcctgagagagctgagccaagaggaagtgcggcaccaccaggatacctggctggccatgcctatctgcagactgagattcatccccaagcctaacggcctgaggcctatcgtgaacatgagctacagcatgggcactagagccctgggcagaagaaagcaggcccagcacttcacccagaggctgaaaaccctgttctccatgctgaactacgagcggacaaagcaccctcatctgatgggctcctctgtgctgggcatgaacgacatctacaggacctggcgggccttcgtgctgagagtcagagcactggaccagacacctagaatgtacttcgtgaaggccgacgtgacaggcgcctacgatgctatccctcagggcaaactggtggaagtggtggccaacatgatcaggcacagcgagtccacctactgcatcagacagtacgccgtcgtgcggagagactctcagggacaagtgcacaagagcttccgcagacaagtgaccacactgagcgatctgcagccctacatgggccagtttctgaagcacctccaggacagcgacgccagcgctctgagaaactctgtggtcatcgagcagtccatctccatgaacgagtccagctccagcctgttcgacttcttcctgcacttcctgcggcacagcgtggtcaagatcggcgacagatgttacacccagtgccagggcatcccacagggaagcagtctgagcacactgctgtgctccctgtgtttcggcgacatggaaaacaagctgttcgccgaagtgcagcgcgacggactgctcctgagatttgtggacgacttcctgctcgtgacccctcacctggatcaggctaagaccttcctgagcaccctggtgcatggcgtgccagagtacggctgcatgatcaacctgcagaaaaccgtggtcaacttccccgtggaacctggcactcttggaggcgctgctccttatcagctgcccgctcattgtctgttcccttggtgcggactgctgctggacacacagaccctggaagtgttctgcgactacagcggctacgcccagaccagcatcaagaccagcctgaccttccagtccgtgttcaaggccggcaagaccatgaggaacaagctgctgagtgtgctgaggctgaagtgccacggcctgtttctggacctgcaagtgaacagcctgcagaccgtgtgcatcaatatctacaagatctttctgctgcaagcctaccggttccacgcctgtgtgattcagctgcctttcgaccagagagtgcggaagaatctgacattctttctgggcatcatcagcagccaggccagctgctgttacgccatcctgaaagtgaagaaccccggcatgaccctgaaggcctctggcagctttccacctgaagctgcccattggctgtgctaccaggctttcctgctgaaactggctgcccacagcgtgatctacaagtgcctgctgggcccactgagaacagcccagaaactgctgtgtcggaagctgcctgaagccacaatgacaatcctgaaggctgccgccgatccagctctgagcaccgacttccagaccatcctggactgagaattcggatccgattcgagcatttaaatacgtggagctcgctgatcagcctcgactgtgccttctagttgccagccatctgttgtttgcccctcccccgtgccttccttgaccctggaaggtgccactcccactgtcctttcctaataaaatgaggaaattgcatcgcattgtctgagtaggtgtcattctattctggggggtggggtggggcaggacagcaagggggaggattgggaagacaatagcaggcatgctggggatgcggtgggctctatggccacgtggatatcgcggccgcaggaacccctagtgatggagttggccactccctctctgcgcgctcgctcgctcactgaggccgggcgaccaaaggtcgcccgacgcccgggctttgcccgggcggcctcagtgagcgagcgagcgcgcagctgcctgcagg

SEQ ID NO: 23 - DNA, 4536 bp, Artificial sequence
  AAV9-TNT-moTert
cctgcaggcagctgcgcgctcgctcgctcactgaggccgcccgggcaaagcccgggcgtcgggcgacctttggtcgcccggcctcagtgagcgagcgagcgcgcagagagggagtggccaactccatcactaggggttcctgcggccgcgatatcctcagtccattaggagccagtagcctggaagatgtctttacccccagcatcagttcaagtggagcagcacataactcttgccctctgccttccaagattctggtgctgagacttatggagtgtcttggaggttgccttctgccccccaaccctgctcccagctggccctcccaggcctgggttgctggcctctgctttatcaggattctcaagagggacagctggtttatgttgcatgactgttccctgcatatctgctctggttttaaatagcttatctgagcagctggaggaccacatgggcttatatggcgtggggtacatgttcctgtagccttgtccctggcacctgccaaaatagcagccaacaccccccacccccaccgccatccccctgccccacccgtcccctgtcgcacattcctccctccgcagggctggctcaccaggccccagcccacatgcctgcttaaagccctctccatcctctgcctcacccagtccccgctgagactgagcagacgcctccaggatctgtcggcaggaattatcgctagcacgcgtgccaccatgacaagagcccctagatgtcctgccgtcagaagcctgctgagaagcagatacagagaagtgtggcccctggccaccttcgtcagaaggcttggacctgaaggcagacggctggttcaacctggcgaccccaagatctacagaaccctggtggctcagtgcctcgtgtgtatgcactggggatctcagccacctcctgccgatctgagctttcaccaggtgtccagcctgaaagaactggtggccagagtggtgcagagactgtgcgagagaaacgagaggaacgtgctggccttcggcttcgagctgctgaatgaagctagaggcggccctcctatggccttcacatctagcgtgcggagctacctgcctaacaccgtgatcgagacactgagagtgtccggcgcttggatgctgctgctgagcagagtgggagatgacctgctggtgtacctgctggctcactgtgccctctatctgctggtgcctcctagctgcgcttaccaagtgtgcggaagccctctgtaccagatctgtgccaccaccgacatctggcctagcgtgtccgcttcctacagacccacaagacccgtgggcagaaactttaccaacctgagattcctgcagcagatcaagagcagctccaggcaagaggcccctaagcctcttgctctgcctagcagaggcaccaagagacacctgagcctgaccagcacaagcgtgccctctgccaagaaagccagatgctaccccgtgcctagagtggaagagggcccacatagacaggtgctgcctacacctagcggcaagagctgggttccatctcctgctagaagccctgaggtgccaacagccgagaaggacctgagcagcaagggcaaagtgtccgacctgtctctgagcggcagcgtgtgttgcaagcacaagcctagcagcaccagcctgctgtccccacctagacagaacgctttccagctgaggccctttatcgagacaagacacttcctgtacagcagaggcgacggccaagagagactgaaccctagcttcctgctgtctaacctgcagcctaacctgaccggcgctagaaggctggtggaaatcatcttcctgggcagcagacccagaaccagcggacctctgtgtagaacccacagactgagcagacggtactggcagatgaggcccctgttccagcagctcctggtcaaccatgccgagtgtcagtatgtgcggctgctgaggtcccactgcagattcagaaccgccaaccagcaagtgacagacgccctgaacacaagccctccacacctgatggatctgctgagactgcacagcagcccctggcaggtctacggctttctgagagcctgtctgtgcaaggtggtgtccgcatctctgtggggcaccagacacaacgagagaagattcttcaagaacctgaagaagttcatcagcctggggaagtacggcaagctgtccctgcaagaactgatgtggaagatgaaggtcgaggactgccactggctgaggtctagccctggcaaggatagagtgcctgccgctgagcacaggctgagagagagaatcctggccacattcctgttctggctgatggacacctacgtggtgcagctgctgcggagcttcttctacatcaccgagagcaccttccagaagaaccggctgttcttctaccgcaagagcgtgtggtccaagctgcagagcatcggcgtcagacagcacctggaaagagtgcgcctgagagagctgagccaagaggaagtgcggcaccaccaggatacctggctggccatgcctatctgcagactgagattcatccccaagcctaacggcctgaggcctatcgtgaacatgagctacagcatgggcactagagccctgggcagaagaaagcaggcccagcacttcacccagaggctgaaaaccctgttctccatgctgaactacgagcggacaaagcaccctcatctgatgggctcctctgtgctgggcatgaacgacatctacaggacctggcgggccttcgtgctgagagtcagagcactggaccagacacctagaatgtacttcgtgaaggccgacgtgacaggcgcctacgatgctatccctcagggcaaactggtggaagtggtggccaacatgatcaggcacagcgagtccacctactgcatcagacagtacgccgtcgtgcggagagactctcagggacaagtgcacaagagcttccgcagacaagtgaccacactgagcgatctgcagccctacatgggccagtttctgaagcacctccaggacagcgacgccagcgctctgagaaactctgtggtcatcgagcagtccatctccatgaacgagtccagctccagcctgttcgacttcttcctgcacttcctgcggcacagcgtggtcaagatcggcgacagatgttacacccagtgccagggcatcccacagggaagcagtctgagcacactgctgtgctccctgtgtttcggcgacatggaaaacaagctgttcgccgaagtgcagcgcgacggactgctcctgagatttgtggacgacttcctgctcgtgacccctcacctggatcaggctaagaccttcctgagcaccctggtgcatggcgtgccagagtacggctgcatgatcaacctgcagaaaaccgtggtcaacttccccgtggaacctggcactcttggaggcgctgctccttatcagctgcccgctcattgtctgttcccttggtgcggactgctgctggacacacagaccctggaagtgttctgcgactacagcggctacgcccagaccagcatcaagaccagcctgaccttccagtccgtgttcaaggccggcaagaccatgaggaacaagctgctgagtgtgctgaggctgaagtgccacggcctgtttctggacctgcaagtgaacagcctgcagaccgtgtgcatcaatatctacaagatctttctgctgcaagcctaccggttccacgcctgtgtgattcagctgcctttcgaccagagagtgcggaagaatctgacattctttctgggcatcatcagcagccaggccagctgctgttacgccatcctgaaagtgaagaaccccggcatgaccctgaaggcctctggcagctttccacctgaagctgcccattggctgtgctaccaggctttcctgctgaaactggctgcccacagcgtgatctacaagtgcctgctgggcccactgagaacagcccagaaactgctgtgtcggaagctgcctgaagccacaatgacaatcctgaaggctgccgccgatccagctctgagcaccgacttccagaccatcctggactgagaattcggatccgattcgagcatttaaatacgtggagctcgctgatcagcctcgactgtgccttctagttgccagccatctgttgtttgcccctcccccgtgccttccttgaccctggaaggtgccactcccactgtcctttcctaataaaatgaggaaattgcatcgcattgtctgagtaggtgtcattctattctggggggtggggtggggcaggacagcaagggggaggattgggaagacaatagcaggcatgctggggatgcggtgggctctatggccacgtggatatcgcggccgcaggaacccctagtgatggagttggccactccctctctgcgcgctcgctcgctcactgaggccgggcgaccaaaggtcgcccgacgcccgggctttgcccgggcggcctcagtgagcgagcgagcgcgcagctgcctgcagg

SEQ ID NO: 24 - DNA, 2027 bp, Artificial Sequence
  AAV9-CMV-null genome and AAV6-CMV-null virus genome
gcgcgctcgctcgctcactgaggccgcccgggcaaagcccgggcgtcgggcgacctttggtcgcccggcctcagtgagcgagcgagcgcgcagagagggagtggccaactccatcactaggggttcctgcggccgcacgcgtggagctagttattaatagtaatcaattacggggtcattagttcatagcccatatatggagttccgcgttacataacttacggtaaatggcccgcctggctgaccgcccaacgacccccgcccattgacgtcaataatgacgtatgttcccatagtaacgtcaatagggactttccattgacgtcaatgggtggagtatttacggtaaactgcccacttggcagtacatcaagtgtatcatatgccaagtacgccccctattgacgtcaatgacggtaaatggcccgcctggcattatgcccagtacatgaccttatgggactttcctacttggcagtacatctacgtattagtcatcgctattaccatggtgatgcggttttggcagtacatcaatgggcgtggatagcggtttgactcacggggatttccaagtctccaccccattgacgtcaatgggagtttgttttgcaccaaaatcaacgggactttccaaaatgtcgtaacaactccgccccattgacgcaaatgggcggtaggcgtgtacggtgggaggtctatataagcagagctcgtttagtgaaccgtcagatcgcctggagacgccatccacgctgttttgacctccatagaagacaccgggaccgatccagcctccgcggattcgaatcccggccgggaacggtgcattggaacgcggattccccgtgccaagagtgacgtaagtaccgcctatagagtctataggcccacaaaaaatgctttcttcttttaatatacttttttgtttatcttatttctaatactttccctaatctctttctttcagggcaataatgatacaatgtatcatgcctctttgcaccattctaaagaataacagtgataatttctgggttaaggcaatagcaatatttctgcatataaatatttctgcatataaattgtaactgatgtaagaggtttcatattgctaatagcagctacaatccagctaccattctgcttttattttatggttgggataaggctggattattctgagtccaagctaggcccttttgctaatcatgttcatacctcttatcttcctcccacagctcctgggcaacgtgctggtctgtgtgctggcccatcactttggcaaagaattgggattcgaacatcgattgaattccccggggatcctctagagtcgacctgcagaagcttgcctcgagcagcgctgctcgagagatctacgggtggcatccctgtgacccctccccagtgcctctcctggccctggaagttgccactccagtgcccaccagccttgtcctaataaaattaagttgcatcattttgtctgactaggtgtccttctataatattatggggtggaggggggtggtatggagcaaggggcaagttgggaagacaacctgtagggcctgcggggtctattgggaaccaagctggagtgcagtggcacaatcttggctcactgcaatctccgcctcctgggttcaagcgattctcctgcctcagcctcccgagttgttgggattccaggcatgcatgaccaggctcagctaatttttgtttttttggtagagacggggtttcaccatattggccaggctggtctccaactcctaatctcaggtgatctacccaccttggcctcccaaattgctgggattacaggcgtgaaccactgctcccttccctgtccttctgattttgtaggtaaccacgtgcggaccgagcggccgcaggaacccctagtgatggagttggccactccctctctgcgcgctcgctcgctcactgaggccgggcgaccaaaggtcgcccgacgcccgggctttgcccgggcggcctcagtgagcgagcgagcgcgc

SEQ ID NO: 25 - DNA, 5320 bp, Artificial Sequence
  AAV9-CMV-mTERT virus genome
cctgcaggcagctgcgcgctcgctcgctcactgaggccgcccgggcaaagcccgggcgtcgggcgacctttggtcgcccggcctcagtgagcgagcgagcgcgcagagagggagtggccaactccatcactaggggttcctgcggccgcacgcgtggagctagttattaatagtaatcaattacggggtcattagttcatagcccatatatggagttccgcgttacataacttacggtaaatggcccgcctggctgaccgcccaacgacccccgcccattgacgtcaataatgacgtatgttcccatagtaacgtcaatagggactttccattgacgtcaatgggtggagtatttacggtaaactgcccacttggcagtacatcaagtgtatcatatgccaagtacgccccctattgacgtcaatgacggtaaatggcccgcctggcattatgcccagtacatgaccttatgggactttcctacttggcagtacatctacgtattagtcatcgctattaccatggtgatgcggttttggcagtacatcaatgggcgtggatagcggtttgactcacggggatttccaagtctccaccccattgacgtcaatgggagtttgttttgcaccaaaatcaacgggactttccaaaatgtcgtaacaactccgccccattgacgcaaatgggcggtaggcgtgtacggtgggaggtctatataagcagagctcgtttagtgaaccgtcagatcgcctggagacgccatccacgctgttttgacctccatagaagacaccgggaccgatccagcctccgcggattcgaatcccggccgggaacggtgcattggaacgcggattccccgtgccaagagtgacgtaagtaccgcctatagagtctataggcccacaaaaaatgctttcttcttttaatatacttttttgtttatcttatttctaatactttccctaatctctttctttcagggcaataatgatacaatgtatcatgcctctttgcaccattctaaagaataacagtgataatttctgggttaaggcaatagcaatatttctgcatataaatatttctgcatataaattgtaactgatgtaagaggtttcatattgctaatagcagctacaatccagctaccattctgcttttattttatggttgggataaggctggattattctgagtccaagctaggcccttttgctaatcatgttcatacctcttatcttcctcccacagctcctgggcaacgtgctggtctgtgtgctggcccatcactttggcaaagaattgggattcgaacatcgattgaattcatgacccgcgctcctcgttgccccgcggtgcgctctctgctgcgcagccgataccgggaggtgtggccgctggcaacctttgtgcggcgcctggggcccgagggcaggcggcttgtgcaacccggggacccgaagatctaccgcactttggttgcccaatgcctagtgtgcatgcactggggctcacagcctccacctgccgacctttccttccaccaggtgtcatccctgaaagagctggtggccagggttgtgcagagactctgcgagcgcaacgagagaaacgtgctggcttttggctttgagctgcttaacgaggccagaggcgggcctcccatggccttcactagtagcgtgcgtagctacttgcccaacactgttattgagaccctgcgtgtcagtggtgcatggatgctactgttgagccgagtgggcgacgacctgctggtctacctgctggcacactgtgctctttatcttctggtgccccccagctgtgcctaccaggtgtgtgggtctcccctgtaccaaatttgtgccaccacggatatctggccctctgtgtccgctagttacaggcccacccgacccgtgggcaggaatttcactaaccttaggttcttacaacagatcaagagcagtagtcgccaggaagcaccgaaacccctggccttgccatctcgaggtacaaagaggcatctgagtctcaccagtacaagtgtgccttcagctaagaaggccagatgctatcctgtcccgagagtggaggagggaccccacaggcaggtgctaccaaccccatcaggcaaatcatgggtgccaagtcctgctcggtcccccgaggtgcctactgcagagaaagatttgtcttctaaaggaaaggtgtctgacctgagtctctctgggtcggtgtgctgtaaacacaagcccagctccacatctctgctgtcaccaccccgccaaaatgcctttcagctcaggccatttattgagaccagacatttcctttactccaggggagatggccaagagcgtctaaacccctcattcctactcagcaacctccagcctaacttgactggggccaggagactggtggagatcatctttctgggctcaaggcctaggacatcaggaccactctgcaggacacaccgtctatcgcgtcgatactggcagatgcggcccctgttccaacagctgctggtgaaccatgcagagtgccaatatgtcagactcctcaggtcacattgcaggtttcgaacagcaaaccaacaggtgacagatgccttgaacaccagcccaccgcacctcatggatttgctccgcctgcacagcagtccctggcaggtatatggttttcttcgggcctgtctctgcaaggtggtgtctgctagtctctggggtaccaggcacaatgagcgccgcttctttaagaacttaaagaagttcatctcgttggggaaatacggcaagctatcactgcaggaactgatgtggaagatgaaagtagaggattgccactggctccgcagcagcccggggaaggaccgtgtccccgctgcagagcaccgtctgaggagaggatcctggctacgttcctgttctggctgatggacacatacgtggtacagctgcttaggtcattcttttacatcacagagagcacattccagaagaacaggctcttcttctaccgtaagagtgtgtggagcaagctgcagagcattggagtcaggcaacaccttgagagagtgcggctacgggagctgtcacaagaggaggtcaggcatcaccaggacacctggctagccatgcccatctgcagactgcgcttcatccccaagcccaacggcctgcggcccattgtgaacatgagttatagcatgggtaccagagctttgggcagaaggaagcaggcccagcatttcacccagcgtctcaagactctcttcagcatgctcaactatgagcggacaaaacatcctcaccttatggggtcttctgtactgggtatgaatgacatctacaggacctggcgggcctttgtgctgcgtgtgcgtgctctggaccagacacccaggatgtactttgttaaggcagatgtgaccggggcctatgatgccatccccccagggtaagctggtggaggttgttgccaatatgatcaggcactcggagagcacgtactgtatccgccagtatgcagtggtccggagagatagccaaggccaagtccacaagtcctttaggagacaggtcaccaccctctctgacctccagccatacatgggccagttccttaagcatctgcaggattcagatgccagtgcactgaggaactccgttgtcatcgagcagagcatctctatgaatgagagcagcagcagcctgtttgacttcttcctgcacttcctgcgtcacagtgtcgtaaagattggtgacaggtgctatacgcagtgccagggcatcccccagggctccagcctatccaccctgctctgcagtctgtgtttcggagacatggagaacaagctgtttgctgaggtgcagcgggatgggttgcttttacgttttgttgatgactttctgttggtgacgcctcacttggaccaagcaaaaaccttcctcagcaccctggtccatggcgttcctgagtatgggtgcatgataaacttgcagaagacagtggtgaacttccctgtggagcctggtaccctgggtggtgcagctccataccagctgcctgctcactgcctgtttccctggtgtggcttgctgctggacactcagactttggaggtgttctgtgactactcaggttatgcccagacctcaattaagacgagcctcaccttccagagtgtcttcaaagctgggaagaccatgcggaacaagctcctgtcggtcttgcggttgaagtgtcacggtctatttctagacttgcaggtgaacagcctccagacagtctgcatcaatatatacaagatcttcctgcttcaggcctacaggttccatgcatgtgtgattcagcttccctttgaccagcgtgttaggaagaacctcacattctttctgggcatcatctccagccaagcatcctgctgctatgctatcctgaaggtcaagaatccaggaatgacactaaaggcctctggctcctttcctcctgaagccgcacattggctctgctaccaggccttcctgctcaagctggctgctcattctgtcatctacaaatgtctcctgggacctctgaggacagcccaaaaactgctgtgccggaagctcccagaggcgacaatgaccatccttaaagctgcagctgacccagccctaagcacagactttcagaccattttggactaaccctgtctccttccgctagatgaacatgggcattgtagcctcagcactcctggatccacgtcacaagagggactggtcagttgtgaggctaggtcatcctccaaacctctgtgtcatgggtggtatgggagattgtcccagtgccttgtttcctgtaacaggcttgatttctttcctgatgccctcagggaggcagatcctatcccttttagtggcagggatccactagcaccagcacatgaggagtgcacccagtgcacatgggcactgggacagtggacaggtgtgagattcctgggccctggagtcttttcacacctaaccatgggagcctgtcccagtacatcagagtgcctcggagatgaaaaaggacatcgagccagtgacctaaattacagcctgaatatactctgaattccccggggatcctctagagtcgacctgcagaagctgtaaccacgtgcggaccgagcggccgcaggaacccctagtgatggagttggccactccctctctgcgcgctcgctcgctcactgaggccgggcgaccaaaggtcgcccgacgcccgggctttgcccgggcggcctcagtgagcgagcgagcgcgcagctgcctgcagg

SEQ ID NO: 26 - DNA, 2831 bp, Artificial Sequence
  AAV-CMV-GFP recombinant adeno-associated virus genome
cctgcaggcagctgcgcgctcgctcgctcactgaggccgcccgggcaaagcccgggcgtcgggcgacctttggtcgcccggcctcagtgagcgagcgagcgcgcagagagggagtggccaactccatcactaggggttcctgcggccgcacgcgtggagctagttattaatagtaatcaattacggggtcattagttcatagcccatatatggagttccgcgttacataacttacggtaaatggcccgcctggctgaccgcccaacgacccccgcccattgacgtcaataatgacgtatgttcccatagtaacgtcaatagggactttccattgacgtcaatgggtggagtatttacggtaaactgcccacttggcagtacatcaagtgtatcatatgccaagtacgccccctattgacgtcaatgacggtaaatggcccgcctggcattatgcccagtacatgaccttatgggactttcctacttggcagtacatctacgtattagtcatcgctattaccatggtgatgcggttttggcagtacatcaatgggcgtggatagcggtttgactcacggggatttccaagtctccaccccattgacgtcaatgggagtttgttttgcaccaaaatcaacgggactttccaaaatgtcgtaacaactccgccccattgacgcaaatgggcggtaggcgtgtacggtgggaggtctatataagcagagctcgtttagtgaaccgtcagatcgcctggagacgccatccacgctgttttgacctccatagaagacaccgggaccgatccagcctccgcggattcgaatcccggccgggaacggtgcattggaacgcggattccccgtgccaagagtgacgtaagtaccgcctatagagtctataggcccacaaaaaatgctttcttcttttaatatacttttttgtttatcttatttctaatactttccctaatctctttctttcagggcaataatgatacaatgtatcatgcctctttgcaccattctaaagaataacagtgataatttctgggttaaggcaatagcaatatttctgcatataaatatttctgcatataaattgtaactgatgtaagaggtttcatattgctaatagcagctacaatccagctaccattctgcttttattttatggttgggataaggctggattattctgagtccaagctaggcccttttgctaatcatgttcatacctcttatcttcctcccacagctcctgggcaacgtgctggtctgtgtgctggcccatcactttggcaaagaattgggattcgaacattcgagcgcaagcttgagctagcgctaccggtcgccaccatggtgagcaagggcgaggagctgttcaccggggtggtgcccatcctggtcgagctggacggcgacgtaaacggccacaagttcagcgtgtccggcgagggcgagggcgatgccacctacggcaagctgaccctgaagttcatctgcaccaccggcaagctgcccgtgccctggcccaccctcgtgaccaccctgacctacggcgtgcagtgcttcagccgctaccccgaccacatgaagcagcacgacttcttcaagtccgccatgcccgaaggctacgtccaggagcgcaccatcttcttcaaggacgacggcaactacaagacccgcgccgaggtgaagttcgagggcgacaccctggtgaaccgcatcgagctgaagggcatcgacttcaaggaggacggcaacatcctggggcacaagctggagtacaactacaacagccacaacgtctatatcatggccgacaagcagaagaacggcatcaaggtgaacttcaagatccgccacaacatcgaggacggcagcgtgcagctcgccgaccactaccagcagaacacccccatcggcgacggccccgtgctgctgcccgacaaccactacctgagcacccagtccgccctgagcaaagaccccaacgagaagcgcgatcacatggtcctgctggagttcgtgaccgccgccgggatcactctcggcatggacgagctgtacaagtccggactcagatctcgagctcaagcttcgaattctgcagtcgacggtaccgcgggcccgggatccaccggatctagataactgatccgcgcgatctacgggtggcatccctgtgacccctccccagtgcctctcctggccctggaagttgccactccagtgcccaccagccttgtcctaataaaattaagttgcatcattttgtctgactaggtgtccttctataatattatggggtggaggggggtggtatggagcaaggggcaagttgggaagacaacctgtagggcctgcggggtctattgggaaccaagctggagtgcagtggcacaatcttggctcactgcaatctccgcctcctgggttcaagcgattctcctgcctcagcctcccgagttgttgggattccaggcatgcatgaccaggctcagctaatttttgtttttttggtagagacggggtttcaccatattggccaggctggtctccaactcctaatctcaggtgatctacccaccttggcctcccaaattgctgggattacaggcgtgaaccactgctcccttccctgtccttctgattttgtaggtaaccacgtgcggaccgagcggccgcaggaacccctagtgatggagttggccactccctctctgcgcgctcgctcgctcactgaggccgggcgaccaaaggtcgcccgacgcccgggctttgcccgggcggcctcagtgagcgagcgagcgcgcagctgcctgcagg

SEQ ID NO: 27 - DNA, 1962 bp, Artificial Sequence
  AAV-SpB-GFP recombinant adeno-associated virus genome
cctgcaggcagctgcgcgctcgctcgctcactgaggccgcccgggcaaagcccgggcgtcgggcgacctttggtcgcccggcctcagtgagcgagcgagcgcgcagagagggagtggccaactccatcactaggggttcctgcggccgcgatatcatagggctgtctgggagccactccagggccacagaaatcttgtctctgactcagggtattttgttttctgttttgtgtaaatgctcttctgactaatgcaaaccatgtgtccatagaaccagaagatttttccaggggaaaaggtaaggaggtggtgagagtgtcctgggtctgcccttccagggcttgccctgggttaagagccaggcaggaagctctcaagagcattgctcaagagtagagggggcctgggaggcccagggaggggatgggaggggaacacccaggctgcccccaaccagatgccctccaccctcctcaacctccctcccacggcctggagaggtgggaccaggtatggaggcttgagagcccctggttggaggaagccacaagtccaggaacatgggagtctgggcagggggcaaaggaggcaggaacaggccatcagccaggacaggtggtaaggcaggcaggagtgttcctgctgggaaaaggtgggatcaagcacctggagggctcttcagagcaaagacaaacactgaggtcgctgccactcctacagagcccccacgccccgcccagctataaggggccatgcaccaagcagggtacccaggctgcagaggtgcgaattcatttaaattctagagccaccatggtgagcaagggcgaggagctgttcaccggggtggtgcccatcctggtcgagctggacggcgacgtaaacggccacaagttcagcgtgtccggcgagggcgagggcgatgccacctacggcaagctgaccctgaagttcatctgcaccaccggcaagctgcccgtgccctggcccaccctcgtgaccaccctgacctacggcgtgcagtgcttcagccgctaccccgaccacatgaagcagcacgacttcttcaagtccgccatgcccgaaggctacgtccaggagcgcaccatcttcttcaaggacgacggcaactacaagacccgcgccgaggtgaagttcgagggcgacaccctggtgaaccgcatcgagctgaagggcatcgacttcaaggaggacggcaacatcctggggcacaagctggagtacaactacaacagccacaacgtctatatcatggccgacaagcagaagaacggcatcaaggtgaacttcaagatccgccacaacatcgaggacggcagcgtgcagctcgccgaccactaccagcagaacacccccatcggcgacggccccgtgctgctgcccgacaaccactacctgagcacccagtccgccctgagcaaagaccccaacgagaagcgcgatcacatggtcctgctggagttcgtgaccgccgccgggatcactctcggcatggacgagctgtacaagtaaactcgagcatttaaatacgtggagctcgctgatcagcctcgactgtgccttctagttgccagccatctgttgtttgcccctcccccgtgccttccttgaccctggaaggtgccactcccactgtcctttcctaataaaatgaggaaattgcatcgcattgtctgagtaggtgtcattctattctggggggtggggtggggcaggacagcaagggggaggattgggaagacaatagcaggcatgctggggatgcggtgggctctatggccacgtggatatcgcggccgcaggaacccctagtgatggagttggccactccctctctgcgcgctcgctcgctcactgaggccgggcgaccaaaggtcgcccgacgcccgggctttgcccgggcggcctcagtgagcgagcgagcgcgcagctgcctgcagg

SEQ ID NO: 28 - DNA, 1214 bp, Artificial Sequence
  AAV6-SpB-null genome and AAV9-SpB-null virus genome
cctgcaggcagctgcgcgctcgctcgctcactgaggccgcccgggcaaagcccgggcgtcgggcgacctttggtcgcccggcctcagtgagcgagcgagcgcgcagagagggagtggccaactccatcactaggggttcctgcggccgcgatatcatagggctgtctgggagccactccagggccacagaaatcttgtctctgactcagggtattttgttttctgttttgtgtaaatgctcttctgactaatgcaaaccatgtgtccatagaaccagaagatttttccaggggaaaaggtaaggaggtggtgagagtgtcctgggtctgcccttccagggcttgccctgggttaagagccaggcaggaagctctcaagagcattgctcaagagtagagggggcctgggaggcccagggaggggatgggaggggaacacccaggctgcccccaaccagatgccctccaccctcctcaacctccctcccacggcctggagaggtgggaccaggtatggaggcttgagagcccctggttggaggaagccacaagtccaggaacatgggagtctgggcagggggcaaaggaggcaggaacaggccatcagccaggacaggtggtaaggcaggcaggagtgttcctgctgggaaaaggtgggatcaagcacctggagggctcttcagagcaaagacaaacactgaggtcgctgccactcctacagagcccccacgccccgcccagctataaggggccatgcaccaagcagggtacccaggctgcagaggtgcgaattcatttaaatacgtggagctcgctgatcagcctcgactgtgccttctagttgccagccatctgttgtttgcccctcccccgtgccttccttgaccctggaaggtgccactcccactgtcctttcctaataaaatgaggaaattgcatcgcattgtctgagtaggtgtcattctattctggggggtggggtggggcaggacagcaagggggaggattgggaagacaatagcaggcatgctggggatgcggtgggctctatggccacgtggatatcgcggccgcaggaacccctagtgatggagttggccactccctctctgcgcgctcgctcgctcactgaggccgggcgaccaaaggtcgcccgacgcccgggctttgcccgggcggcctcagtgagcgagcgagcgcgcagctgcctgcagg

SEQ ID NO: 29 - DNA, 19 bp, Artificial Sequence
  Set 1 Forward
tagccctggcaaggataga

SEQ ID NO: 30 - DNA, 22 bp, Artificial Sequence
  Set 1 Reverse
gctctcggtgatgtagaagaag

SEQ ID NO: 31 - DNA, 21 bp, Artificial Sequence
  Set 2 Forward
caccagacacaacgagagaag

SEQ ID NO: 32 - DNA, 22 bp, Artificial Sequence
  Set 2 reverse
ctcgaccttcatcttccacatc

SEQ ID NO: 33 - DNA, 18 bp, Artificial Sequence
  GFP forward primer
agctggacggcgacgtaa

SEQ ID NO: 34 - DNA, 22 bp, Artificial Sequence
  GFP reverse primer
gtgcagatgaacttcagggtca

SEQ ID NO: 35 - DNA, 21 bp, Artificial Sequence
  moTERT forward primer
caccagacacaacgagagaag

SEQ ID NO: 36 - DNA, 22 bp, Artificial Sequence
  moTERT reverse primer
ctcgaccttcatcttccacatc

SEQ ID NO: 37 - DNA, 22 bp, Artificial Sequence
  FAM-Probe
agggacagcttgccgtacttcc

SEQ ID NO: 38 - DNA, 21 bp, Artificial Sequence
  ITR2 forward primer
ggaacccctagtgatggagtt

SEQ ID NO: 39 - DNA, 16 bp, Artificial Sequence
  ITR2 reverse primer
cggcctcagtgagcga

SEQ ID NO: 40 - DNA, 21 bp, Artificial Sequence
  HEX-Probe
cactccctctctgcgcgctcg

SEQ ID NO: 41 - DNA, 21 bp, Artificial Sequence
  moTERT forward primer
ggaagtgttctgcgactacag

SEQ ID NO: 42 - DNA, 21 bp, Artificial Sequence
  moTERT reverse primer
cagcttgttcctcatggtctt

SEQ ID NO: 43 - DNA, 25 bp, Artificial Sequence
  probe /56FAM
  misc_feature 10: /note="n= ZEN"
ctacgcccangaccagcatcaagac

SEQ ID NO: 44 - DNA, 20 bp, Artificial Sequence
  hRplp0 forward primer
cagacagacactggcaacat

SEQ ID NO: 45 - DNA, 20 bp, Artificial Sequence
  hRplp0 reverse primer
gcagcatctacaaccctgaa

SEQ ID NO: 46 - DNA, 25 bp, Artificial Sequence
  Probe: /5HEX
  misc_feature 10: /note="n=ZEN"
aactctgcanttctcgcttcctgga